European Patent Specification EP 2 862 875 B1, published September 6, 2023. Title: ANTIGEN BINDING MOLECULES COMPRISING MODIFIED FC REGIONS. Applicant: CHUGAI SEIYAKU KABUSHIKI KAISHA. The sequence listing filed with the application follows.

SEQUENCE LISTING (54 sequences)

SEQ ID NO: 1 - protein, 115 aa, Artificial
  An artificially synthesized peptide sequence
QVQLVQSGAEVKKPGASVTVSCKASGYTFTDYEMHWIRQPPGEGLEWIGAIDPKTGDTAYSESFQDRVTLTADKSTSTAYMELSSLTSEDTAVYYCTRFYSYTYWGQGTLVTVSS

SEQ ID NO: 2 - protein, 443 aa, Artificial
  An artificially synthesized peptide sequence
QVQLVQSGAEVKKPGASVTVSCKASGYTFTDYEMHWIRQPPGEGLEWIGAIDPKTGDTAYSESFQDRVTLTADKSTSTAYMELSSLTSEDTAVYYCTRFYSYTYWGQGTLVTVSSASTKGPSVFPLAPSSKSTSGGTAALGCLVKDYFPEPVTVSWNSGALTSGVHTFPAVLQSSGLYSLSSVVTVPSSSLGTQTYICNVNHKPSNTKVDKKVEPKSCDKTHTCPPCPAPELLGGPSVFLFPPKPKDTLMISRTPEVTCVVVDVSHEDPEVKFNWYVDGVEVHNAKTKPREEQYNSTYRVVSVLTVLHQDWLNGKEYKCKVSNKALPAPIEKTISKAKGQPREPQVYTLPPSRDELTKNQVSLTCLVKGFYPSDIAVEWESNGQPENNYKTTPPVLDSDGSFFLYSKLTVDKSRWQQGNVFSCSVMHEALHNHYTQKSLSLSP

SEQ ID NO: 3 - protein, 443 aa, Artificial
  An artificially synthesized peptide sequence
QVQLVQSGAEVKKPGASVTVSCKASGYTFTDYEMHWIRQPPGEGLEWIGAIDPKTGDTAYSESFQDRVTLTADKSTSTAYMELSSLTSEDTAVYYCTRFYSYTYWGQGTLVTVSSASTKGPSVFPLAPSSKSTSGGTAALGCLVKDYFPEPVTVSWNSGALTSGVHTFPAVLQSSGLYSLSSVVTVPSSSLGTQTYICNVNHKPSNTKVDKKVEPKSCDKTHTCPPCPAPELLGGPSVFLFPPKPKDTLMISRTPEVTCVVVDVSHEDPEVKFNWYVDGVEVHNAKTKPREEQYNSTYRVVSVLTVLHQDWLNGKEYKCKVSNKALPAPIEKTISKAKGQPREPQVYTLPPSRKELTKNQVSLTCLVKGFYPSDIAVEWESNGQPENNYKTTPPVLDSDGSFFLYSKLTVDKSRWQQGNVFSCSVMHEALHNRYTQKSLSLSP

SEQ ID NO: 4 - protein, 443 aa, Artificial
  An artificially synthesized peptide sequence
QVQLVQSGAEVKKPGASVTVSCKASGYTFTDYEMHWIRQPPGEGLEWIGAIDPKTGDTAYSESFQDRVTLTADKSTSTAYMELSSLTSEDTAVYYCTRFYSYTYWGQGTLVTVSSASTKGPSVFPLAPSSKSTSGGTAALGCLVKDYFPEPVTVSWNSGALTSGVHTFPAVLQSSGLYSLSSVVTVPSSSLGTQTYICNVNHKPSNTKVDKKVEPKSCDKTHTCPPCPAPELLGGPSVFLFPPKPKDTLMISRTPEVTCVVVDVSHEDPEVKFNWYVDGVEVHNAKTKPREEQYNSTYRVVSVLTVLHQDWLNGKEYKCKVSNKALPAPIEKTISKAKGQPREPQVYTLPPSRDELTKNQVSLTCLVKGFYPSDIAVEWESNGQPENNYKTTPPVLDSDGSFFLYSKLTVDKSRWQQGNVFSCSVMHEALHNHYTQESLSLSP

SEQ ID NO: 5 - protein, 219 aa, Artificial
  An artificially synthesized peptide sequence
DIVMTQSPLSLPVTPGEPASISCQASESLVHSNRNTYLHWYLQKPGQSPQLLIYKVSNRFSGVPDRFSGSGSGTDFTLKISRVEAEDVGVYYCSQNTHVPPTFGQGTKVEIERTVAAPSVFIFPPSDEQLKSGTASVVCLLNNFYPREAKVQWKVDNALQSGNSQESVTEQDSKDSTYSLSSTLTLSKADYEKHKVYACEVTHQGLSSPVTKSFNRGEC

SEQ ID NO: 6 - protein, 443 aa, Artificial
  An artificially synthesized peptide sequence
QVQLVQSGAEVKKPGASVTVSCKASGYTFTDYEMHWIRQPPGEGLEWIGAIDPKTGDTAYSESFQDRVTLTADKSTSTAYMELSSLTSEDTAVYYCTRFYSYTYWGQGTLVTVSSASTKGPSVFPLAPSSKSTSGGTAALGCLVKDYFPEPVTVSWNSGALTSGVHTFPAVLQSSGLYSLSSVVTVPSSSLGTQTYICNVNHKPSNTKVDKKVEPKSCDKTHTCPPCPAPELLGGPDVFLFPPKPKDTLMISRTPEVTCVVVDVSHEDPEVKFNWYVDGVEVHNAKTKPREEQYNSTYRVVSVLTVLHQDWLNGKEYKCKVSNKALPLPEEKTISKAKGQPREPQVYTLPPSRKELTKNQVSLTCLVKGFYPSDIAVEWESNGQPENNYKTTPPVLDSDGSFFLYSKLTVDKSRWQQGNVFSCSVMHEALHNRYTQKSLSLSP

SEQ ID NO: 7 - protein, 443 aa, Artificial
  An artificially synthesized peptide sequence
QVQLVQSGAEVKKPGASVTVSCKASGYTFTDYEMHWIRQPPGEGLEWIGAIDPKTGDTAYSESFQDRVTLTADKSTSTAYMELSSLTSEDTAVYYCTRFYSYTYWGQGTLVTVSSASTKGPSVFPLAPSSKSTSGGTAALGCLVKDYFPEPVTVSWNSGALTSGVHTFPAVLQSSGLYSLSSVVTVPSSSLGTQTYICNVNHKPSNTKVDKKVEPKSCDKTHTCPPCPAPELLGGPDVFLFPPKPKDTLMISRTPEVTCVVVDVSHEDPEVKFNWYVDGVEVHNAKTKPREEQYNSTYRVVSVLTVLHQDWLNGKEYKCKVSNKALPLPEEKTISKAKGQPREPQVYTLPPSRDELTKNQVSLTCLVKGFYPSDIAVEWESNGQPENNYKTTPPVLDSDGSFFLYSKLTVDKSRWQQGNVFSCSVMHEALHNHYTQESLSLSP

SEQ ID NO: 8 - protein, 443 aa, Artificial
  An artificially synthesized peptide sequence
QVQLVQSGAEVKKPGASVTVSCKASGYTFTDYEMHWIRQPPGEGLEWIGAIDPKTGDTAYSESFQDRVTLTADKSTSTAYMELSSLTSEDTAVYYCTRFYSYTYWGQGTLVTVSSASTKGPSVFPLAPSSKSTSGGTAALGCLVKDYFPEPVTVSWNSGALTSGVHTFPAVLQSSGLYSLSSVVTVPSSSLGTQTYICNVNHKPSNTKVDKKVEPKSCDKTHTCPPCPAPEYLWGPSVFLFPPKPKDTLMISRTPEVTCVVVDVSHEDPEVKFNWYVDGVEVHNAKTKPREEQYNATYRVVSVLTVLHQDWLNGKEYKCKVSNKALPAPIEKTISKAKGQPREPQVYTLPPSRKELTKNQVSLTCLVKGFYPSDIAVEWESNGQPENNYKTTPPVLDSDGSFFLYSKLTVDKSRWQQGNVFSCSVMHEALHNRYTQKSLSLSP

SEQ ID NO: 9 - protein, 443 aa, Artificial
  An artificially synthesized peptide sequence
QVQLVQSGAEVKKPGASVTVSCKASGYTFTDYEMHWIRQPPGEGLEWIGAIDPKTGDTAYSESFQDRVTLTADKSTSTAYMELSSLTSEDTAVYYCTRFYSYTYWGQGTLVTVSSASTKGPSVFPLAPSSKSTSGGTAALGCLVKDYFPEPVTVSWNSGALTSGVHTFPAVLQSSGLYSLSSVVTVPSSSLGTQTYICNVNHKPSNTKVDKKVEPKSCDKTHTCPPCPAPEYLWGPSVFLFPPKPKDTLMISRTPEVTCVVVDVSHEDPEVKFNWYVDGVEVHNAKTKPREEQYNATYRVVSVLTVLHQDWLNGKEYKCKVSNKALPAPIEKTISKAKGQPREPQVYTLPPSRDELTKNQVSLTCLVKGFYPSDIAVEWESNGQPENNYKTTPPVLDSDGSFFLYSKLTVDKSRWQQGNVFSCSVMHEALHNHYTQESLSLSP

SEQ ID NO: 10 - protein, 116 aa, Artificial
  An artificially synthesized peptide sequence
QDQLVQSGAEVKKPGASVKVSCKASGFNIKDTYIQWVRQAPGQGLEWMGRIDPLRKQTKYREKFEGRVTITADTSTNTAYMELSSLRSEDTAVYYCVRSGREFDYWGQGTLVTVSS

SEQ ID NO: 11 - protein, 213 aa, Artificial
  An artificially synthesized peptide sequence
DIQMTQSPSSLSASVGDRVTITCRASQDIHKYIAWYQQKPGQAPRLLIQYTSTLQPGVPSRFSGSGSGTDYTFTISSLQPEDIATYYCLQYEQLRTFGGGTKVEIKRTVAAPSVFIFPPSDEQLKSGTASVVCLLNNFYPREAKVQWKVDNALQSGNSQESVTEQDSKDSTYSLSSTLTLSKADYEKHKVYACEVTHQGLSSPVTKSFNRGEC

SEQ ID NO: 12 - protein, 444 aa, Artificial
  An artificially synthesized peptide sequence
QDQLVQSGAEVKKPGASVKVSCKASGFNIKDTYIQWVRQAPGQGLEWMGRIDPLRKQTKYREKFEGRVTITADTSTNTAYMELSSLRSEDTAVYYCVRSGREFDYWGQGTLVTVSSASTKGPSVFPLAPSSKSTSGGTAALGCLVKDYFPEPVTVSWNSGALTSGVHTFPAVLQSSGLYSLSSVVTVPSSSLGTQTYICNVNHKPSNTKVDKKVEPKSCDKTHTCPPCPAPELLGGPSVFLFPPKPKDTLMISRTPEVTCVVVDVSHEDPEVKFNWYVDGVEVHNAKTKPREEQYNSTYRVVSVLTVLHQDWLNGKEYKCKVSNKALPAPIEKTISKAKGQPREPQVYTLPPSRDELTKNQVSLTCLVKGFYPSDIAVEWESNGQPENNYKTTPPVLDSDGSFFLYSKLTVDKSRWQQGNVFSCSVMHEALHNHYTQKSLSLSP

SEQ ID NO: 13 - protein, 444 aa, Artificial
  An artificially synthesized peptide sequence
QDQLVQSGAEVKKPGASVKVSCKASGFNIKDTYIQWVRQAPGQGLEWMGRIDPLRKQTKYREKFEGRVTITADTSTNTAYMELSSLRSEDTAVYYCVRSGREFDYWGQGTLVTVSSASTKGPSVFPLAPSSKSTSGGTAALGCLVKDYFPEPVTVSWNSGALTSGVHTFPAVLQSSGLYSLSSVVTVPSSSLGTQTYICNVNHKPSNTKVDKKVEPKSCDKTHTCPPCPAPELLGGPSVFLFPPKPKDTLMISRTPEVTCVVVDVSHEDPEVKFNWYVDGVEVHNAKTKPREEQYNSTYRVVSVLTVLHQDWLNGKEYKCKVSNKALPAPIEKTISKAKGQPREPQVCTLPPSRDELTKNQVSLWCLVKGFYPSDIAVEWESNGQPENNYKTTPPVLDSDGSFFLYSKLTVDKSRWQQGNVFSCSVMHEALHNHYTQKSLSLSP

SEQ ID NO: 14 - protein, 444 aa, Artificial
  An artificially synthesized peptide sequence
QDQLVQSGAEVKKPGASVKVSCKASGFNIKDTYIQWVRQAPGQGLEWMGRIDPLRKQTKYREKFEGRVTITADTSTNTAYMELSSLRSEDTAVYYCVRSGREFDYWGQGTLVTVSSASTKGPSVFPLAPSSKSTSGGTAALGCLVKDYFPEPVTVSWNSGALTSGVHTFPAVLQSSGLYSLSSVVTVPSSSLGTQTYICNVNHKPSNTKVDKKVEPKSCDKTHTCPPCPAPELLGGPSVFLFPPKPKDTLMISRTPEVTCVVVDVSHEDPEVKFNWYVDGVEVHNAKTKPREEQYNSTYRVVSVLTVLHQDWLNGKEYKCKVSNKALPAPIEKTISKAKGQPREPQVYTLPPSRCELTKNQVSLSCAVKGFYPSDIAVEWESNGQPENNYKTTPPVLDSDGSFFLVSKLTVDKSRWQQGNVFSCSVMHEALHNHYTQKSLSLSP

SEQ ID NO: 15 - protein, 444 aa, Artificial
  An artificially synthesized peptide sequence
QDQLVQSGAEVKKPGASVKVSCKASGFNIKDTYIQWVRQAPGQGLEWMGRIDPLRKQTKYREKFEGRVTITADTSTNTAYMELSSLRSEDTAVYYCVRSGREFDYWGQGTLVTVSSASTKGPSVFPLAPSSKSTSGGTAALGCLVKDYFPEPVTVSWNSGALTSGVHTFPAVLQSSGLYSLSSVVTVPSSSLGTQTYICNVNHKPSNTKVDKKVEPKSCDKTHTCPPCPAPELLGGPDVFLFPPKPKDTLMISRTPEVTCVVVDVSHEDPEVKFNWYVDGVEVHNAKTKPREEQYNSTYRVVSVLTVLHQDWLNGKEYKCKVSNKALPLPEEKTISKAKGQPREPQVCTLPPSRDELTKNQVSLWCLVKGFYPSDIAVEWESNGQPENNYKTTPPVLDSDGSFFLYSKLTVDKSRWQQGNVFSCSVMHEALHNHYTQKSLSLSP

SEQ ID NO: 16 - protein, 444 aa, Artificial
  An artificially synthesized peptide sequence
QDQLVQSGAEVKKPGASVKVSCKASGFNIKDTYIQWVRQAPGQGLEWMGRIDPLRKQTKYREKFEGRVTITADTSTNTAYMELSSLRSEDTAVYYCVRSGREFDYWGQGTLVTVSSASTKGPSVFPLAPSSKSTSGGTAALGCLVKDYFPEPVTVSWNSGALTSGVHTFPAVLQSSGLYSLSSVVTVPSSSLGTQTYICNVNHKPSNTKVDKKVEPKSCDKTHTCPPCPAPELLGGPDVFLFPPKPKDTLMISRTPEVTCVVVDVSHEDPEVKFNWYVDGVEVHNAKTKPREEQYNSTYRVVSVLTVLHQDWLNGKEYKCKVSNKALPLPEEKTISKAKGQPREPQVYTLPPSRCELTKNQVSLSCAVKGFYPSDIAVEWESNGQPENNYKTTPPVLDSDGSFFLVSKLTVDKSRWQQGNVFSCSVMHEALHNHYTQKSLSLSP

SEQ ID NO: 17 - protein, 444 aa, Artificial
  An artificially synthesized peptide sequence
QDQLVQSGAEVKKPGASVKVSCKASGFNIKDTYIQWVRQAPGQGLEWMGRIDPLRKQTKYREKFEGRVTITADTSTNTAYMELSSLRSEDTAVYYCVRSGREFDYWGQGTLVTVSSASTKGPSVFPLAPSSKSTSGGTAALGCLVKDYFPEPVTVSWNSGALTSGVHTFPAVLQSSGLYSLSSVVTVPSSSLGTQTYICNVNHKPSNTKVDKKVEPKSCDKTHTCPPCPAPEYYWGPSVFLFPPKPKDTLMISRTPEVTCVVVDVSDEDPEVKFNWYVDGVEVHNAKTKPREEQYNATYRVVSVLTVLHQDWLNGKEYKCKVSNKALPAPIEKTISKAKGQPREPQVCTLPPSRDELTKNQVSLWCLVKGFYPSDIAVEWESNGQPENNYKTTPPVLDSDGSFFLYSKLTVDKSRWQQGNVFSCSVMHEALHNHYTQKSLSLSP

SEQ ID NO: 18 - protein, 444 aa, Artificial
  An artificially synthesized peptide sequence
QDQLVQSGAEVKKPGASVKVSCKASGFNIKDTYIQWVRQAPGQGLEWMGRIDPLRKQTKYREKFEGRVTITADTSTNTAYMELSSLRSEDTAVYYCVRSGREFDYWGQGTLVTVSSASTKGPSVFPLAPSSKSTSGGTAALGCLVKDYFPEPVTVSWNSGALTSGVHTFPAVLQSSGLYSLSSVVTVPSSSLGTQTYICNVNHKPSNTKVDKKVEPKSCDKTHTCPPCPAPELLGGPSVFLFPPKPKDTLMISRTPEVTCVVVDVSHEDPEVKFNWYVDGVEVHNAKTKPREEQYNSTYRVVSVLTVLHQDWLNGKEYKCKVSNDALPMPIEETISKAKGQPREPQVYTLPPSRCELTKNQVSLSCAVKGFYPSDIAVEWESNGQPENNYKTTPPVLDSDGSFFLVSKLTVDKSRWQQGNVFSCSVMHEALHNHYTQKSLSLSP

SEQ ID NO: 19 - protein, 444 aa, Artificial
  An artificially synthesized peptide sequence
QDQLVQSGAEVKKPGASVKVSCKASGFNIKDTYIQWVRQAPGQGLEWMGRIDPLRKQTKYREKFEGRVTITADTSTNTAYMELSSLRSEDTAVYYCVRSGREFDYWGQGTLVTVSSASTKGPSVFPLAPSSKSTSGGTAALGCLVKDYFPEPVTVSWNSGALTSGVHTFPAVLQSSGLYSLSSVVTVPSSSLGTQTYICNVNHKPSNTKVDKKVEPKSCDKTHTCPPCPAPEYYWGPSVFLFPPKPKDTLMISRTPEVTCVVVDVSDEDPEVKFNWYVDGVEVHNAKTKPREEQYNATYRVVSVLTVLHQDWLNGKEYKCKVSNKALPAPIEKTISKAKGQPREPQVYTLPPSRCELTKNQVSLSCAVKGFYPSDIAVEWESNGQPENNYKTTPPVLDSDGSFFLVSKLTVDKSRWQQGNVFSCSVMHEALHNHYTQKSLSLSP

SEQ ID NO: 20 - protein, 444 aa, Artificial
  An artificially synthesized peptide sequence
QDQLVQSGAEVKKPGASVKVSCKASGFNIKDTYIQWVRQAPGQGLEWMGRIDPLRKQTKYREKFEGRVTITADTSTNTAYMELSSLRSEDTAVYYCVRSGREFDYWGQGTLVTVSSASTKGPSVFPLAPSSKSTSGGTAALGCLVKDYFPEPVTVSWNSGALTSGVHTFPAVLQSSGLYSLSSVVTVPSSSLGTQTYICNVNHKPSNTKVDKKVEPKSCDKTHTCPPCPAPELLGGPSVFLFPPKPKDTLMISRTPEVTCVVVDVSHEDPEVKFNWYVDGVEVHNAKTKPREEQYNSTYRVVSVLTVLHQDWLNGKEYKCKVSNDALPMPIEETISKAKGQPREPQVCTLPPSRDELTKNQVSLWCLVKGFYPSDIAVEWESNGQPENNYKTTPPVLDSDGSFFLYSKLTVDKSRWQQGNVFSCSVMHEALHNHYTQKSLSLSP

SEQ ID NO: 21 - protein, 444 aa, Artificial
  An artificially synthesized peptide sequence
QDQLVQSGAEVKKPGASVKVSCKASGFNIKDTYIQWVRQAPGQGLEWMGRIDPLRKQTKYREKFEGRVTITADTSTNTAYMELSSLRSEDTAVYYCVRSGREFDYWGQGTLVTVSSASTKGPSVFPLAPSSKSTSGGTAALGCLVKDYFPEPVTVSWNSGALTSGVHTFPAVLQSSGLYSLSSVVTVPSSSLGTQTYICNVNHKPSNTKVDKKVEPKSCDKTHTCPPCPAPEYQWGPMVFLFPPKPKDTLMISRTPEVTCVVVDVSDEEPEVKFNWYVDGVEVHNAKTKPREEQYNATYRVVSVLTVLHQDWLNGKEYKCKVSNKALPAPIEKTISKAKGQPREPQVCTLPPSRDELTKNQVSLWCLVKGFYPSDIAVEWESNGQPENNYKTTPPVLDSDGSFFLYSKLTVDKSRWQQGNVFSCSVMHEALHNHYTQKSLSLSP

SEQ ID NO: 22 - protein, 444 aa, Artificial
  An artificially synthesized peptide sequence
QDQLVQSGAEVKKPGASVKVSCKASGFNIKDTYIQWVRQAPGQGLEWMGRIDPLRKQTKYREKFEGRVTITADTSTNTAYMELSSLRSEDTAVYYCVRSGREFDYWGQGTLVTVSSASTKGPSVFPLAPSSKSTSGGTAALGCLVKDYFPEPVTVSWNSGALTSGVHTFPAVLQSSGLYSLSSVVTVPSSSLGTQTYICNVNHKPSNTKVDKKVEPKSCDKTHTCPPCPAPELLGGPSVFLFPPKPKDTLMISRTPEVTCVVVDVSHEEPEVKFNWYVDGVEVHNAKTKPREEQYNSTYRVVSVLTVLHQDWLNGKEYKCKVSNDALPMPIEETISKAKGQPREPQVYTLPPSRCELTKNQVSLSCAVKGFYPSDIAVEWESNGQPENNYKTTPPVLDSDGSFFLVSKLTVDKSRWQQGNVFSCSVMHEALHNHYTQKSLSLSP

SEQ ID NO: 23 - protein, 444 aa, Artificial
  An artificially synthesized peptide sequence
QDQLVQSGAEVKKPGASVKVSCKASGFNIKDTYIQWVRQAPGQGLEWMGRIDPLRKQTKYREKFEGRVTITADTSTNTAYMELSSLRSEDTAVYYCVRSGREFDYWGQGTLVTVSSASTKGPSVFPLAPSSKSTSGGTAALGCLVKDYFPEPVTVSWNSGALTSGVHTFPAVLQSSGLYSLSSVVTVPSSSLGTQTYICNVNHKPSNTKVDKKVEPKSCDKTHTCPPCPAPELLGGPSVFLFPPKPKDTLMISRTPEVTCVVVDVGGSGGSVKFNWYVDGVEVHNAKTKPREEQYNSTYRVVSVLTVLHQDWLNGKEYKCKVSNDALPMPIEETISKAKGQPREPQVYTLPPSRCELTKNQVSLSCAVKGFYPSDIAVEWESNGQPENNYKTTPPVLDSDGSFFLVSKLTVDKSRWQQGNVFSCSVMHEALHNHYTQKSLSLSP

SEQ ID NO: 24 - protein, 450 aa, Artificial
  An artificially synthesized peptide sequence
QDQLVQSGAEVKKPGASVKVSCKASGFNIKDTYIQWVRQAPGQGLEWMGRIDPLRKQTKYREKFEGRVTITADTSTNTAYMELSSLRSEDTAVYYCVRSGREFDYWGQGTLVTVSSASTKGPSVFPLAPSSKSTSGGTAALGCLVKDYFPEPVTVSWNSGALTSGVHTFPAVLQSSGLYSLSSVVTVPSSSLGTQTYICNVNHKPSNTKVDKKVEPKSCDKTHTCPPCPAPELLGGPSVFLFPPKPKDTLMISRTPEVTCVVVDVGGGSGGGSGGGSVKFNWYVDGVEVHNAKTKPREEQYNSTYRVVSVLTVLHQDWLNGKEYKCKVSNDALPMPIEETISKAKGQPREPQVYTLPPSRCELTKNQVSLSCAVKGFYPSDIAVEWESNGQPENNYKTTPPVLDSDGSFFLVSKLTVDKSRWQQGNVFSCSVMHEALHNHYTQKSLSLSP

SEQ ID NO: 25 - protein, 450 aa, Artificial; identical to SEQ ID NO: 24
  An artificially synthesized peptide sequence

SEQ ID NO: 26 - protein, 447 aa, Artificial
  An artificially synthesized peptide sequence
QDQLVQSGAEVKKPGASVKVSCKASGFNIKDTYIQWVRQAPGQGLEWMGRIDPLRKQTKYREKFEGRVTITADTSTNTAYMELSSLRSEDTAVYYCVRSGREFDYWGQGTLVTVSSASTKGPSVFPLAPSSKSTSGGTAALGCLVKDYFPEPVTVSWNSGALTSGVHTFPAVLQSSGLYSLSSVVTVPSSSLGTQTYICNVNHKPSNTKVDKKVEPKSCDKTHTCPPCPAPELLGGPSVFLFPPKPKDTLMISRTPEVTCVVVDVSHGGSEEPEVKFNWYVDGVEVHNAKTKPREEQYNSTYRVVSVLTVLHQDWLNGKEYKCKVSNDALPMPIEETISKAKGQPREPQVYTLPPSRCELTKNQVSLSCAVKGFYPSDIAVEWESNGQPENNYKTTPPVLDSDGSFFLVSKLTVDKSRWQQGNVFSCSVMHEALHNHYTQKSLSLSP

SEQ ID NO: 27 - protein, 450 aa, Artificial
  An artificially synthesized peptide sequence
QDQLVQSGAEVKKPGASVKVSCKASGFNIKDTYIQWVRQAPGQGLEWMGRIDPLRKQTKYREKFEGRVTITADTSTNTAYMELSSLRSEDTAVYYCVRSGREFDYWGQGTLVTVSSASTKGPSVFPLAPSSKSTSGGTAALGCLVKDYFPEPVTVSWNSGALTSGVHTFPAVLQSSGLYSLSSVVTVPSSSLGTQTYICNVNHKPSNTKVDKKVEPKSCDKTHTCPPCPAPELLGGPSVFLFPPKPKDTLMISRTPEVTCVVVDVSHGGSGGSEEPEVKFNWYVDGVEVHNAKTKPREEQYNSTYRVVSVLTVLHQDWLNGKEYKCKVSNDALPMPIEETISKAKGQPREPQVYTLPPSRCELTKNQVSLSCAVKGFYPSDIAVEWESNGQPENNYKTTPPVLDSDGSFFLVSKLTVDKSRWQQGNVFSCSVMHEALHNHYTQKSLSLSP

SEQ ID NO: 28 - protein, 453 aa, Artificial
  An artificially synthesized peptide sequence
QDQLVQSGAEVKKPGASVKVSCKASGFNIKDTYIQWVRQAPGQGLEWMGRIDPLRKQTKYREKFEGRVTITADTSTNTAYMELSSLRSEDTAVYYCVRSGREFDYWGQGTLVTVSSASTKGPSVFPLAPSSKSTSGGTAALGCLVKDYFPEPVTVSWNSGALTSGVHTFPAVLQSSGLYSLSSVVTVPSSSLGTQTYICNVNHKPSNTKVDKKVEPKSCDKTHTCPPCPAPELLGGPSVFLFPPKPKDTLMISRTPEVTCVVVDVSHGGSGGSGGSEEPEVKFNWYVDGVEVHNAKTKPREEQYNSTYRVVSVLTVLHQDWLNGKEYKCKVSNDALPMPIEETISKAKGQPREPQVYTLPPSRCELTKNQVSLSCAVKGFYPSDIAVEWESNGQPENNYKTTPPVLDSDGSFFLVSKLTVDKSRWQQGNVFSCSVMHEALHNHYTQKSLSLSP

SEQ ID NO: 29 - protein, 447 aa, Artificial
  An artificially synthesized peptide sequence
QDQLVQSGAEVKKPGASVKVSCKASGFNIKDTYIQWVRQAPGQGLEWMGRIDPLRKQTKYREKFEGRVTITADTSTNTAYMELSSLRSEDTAVYYCVRSGREFDYWGQGTLVTVSSASTKGPSVFPLAPSSKSTSGGTAALGCLVKDYFPEPVTVSWNSGALTSGVHTFPAVLQSSGLYSLSSVVTVPSSSLGTQTYICNVNHKPSNTKVDKKVEPKSCDKTHTCPPCPAPELLGGPSVFLFPPKPKDTLMISRTPEVTCVVVDVSHEEPEVKFNWYVDGVEVHNAKTKPREEQYNSTGGSYRVVSVLTVLHQDWLNGKEYKCKVSNDALPMPIEETISKAKGQPREPQVYTLPPSRCELTKNQVSLSCAVKGFYPSDIAVEWESNGQPENNYKTTPPVLDSDGSFFLVSKLTVDKSRWQQGNVFSCSVMHEALHNHYTQKSLSLSP

SEQ ID NO: 30 - protein, 450 aa, Artificial
  An artificially synthesized peptide sequence
QDQLVQSGAEVKKPGASVKVSCKASGFNIKDTYIQWVRQAPGQGLEWMGRIDPLRKQTKYREKFEGRVTITADTSTNTAYMELSSLRSEDTAVYYCVRSGREFDYWGQGTLVTVSSASTKGPSVFPLAPSSKSTSGGTAALGCLVKDYFPEPVTVSWNSGALTSGVHTFPAVLQSSGLYSLSSVVTVPSSSLGTQTYICNVNHKPSNTKVDKKVEPKSCDKTHTCPPCPAPELLGGPSVFLFPPKPKDTLMISRTPEVTCVVVDVSHEEPEVKFNWYVDGVEVHNAKTKPREEQYNSTGGSGGSYRVVSVLTVLHQDWLNGKEYKCKVSNDALPMPIEETISKAKGQPREPQVYTLPPSRCELTKNQVSLSCAVKGFYPSDIAVEWESNGQPENNYKTTPPVLDSDGSFFLVSKLTVDKSRWQQGNVFSCSVMHEALHNHYTQKSLSLSP

SEQ ID NO: 31 - protein, 453 aa, Artificial
  An artificially synthesized peptide sequence
QDQLVQSGAEVKKPGASVKVSCKASGFNIKDTYIQWVRQAPGQGLEWMGRIDPLRKQTKYREKFEGRVTITADTSTNTAYMELSSLRSEDTAVYYCVRSGREFDYWGQGTLVTVSSASTKGPSVFPLAPSSKSTSGGTAALGCLVKDYFPEPVTVSWNSGALTSGVHTFPAVLQSSGLYSLSSVVTVPSSSLGTQTYICNVNHKPSNTKVDKKVEPKSCDKTHTCPPCPAPELLGGPSVFLFPPKPKDTLMISRTPEVTCVVVDVSHEEPEVKFNWYVDGVEVHNAKTKPREEQYNSTGGSGGSGGSYRVVSVLTVLHQDWLNGKEYKCKVSNDALPMPIEETISKAKGQPREPQVYTLPPSRCELTKNQVSLSCAVKGFYPSDIAVEWESNGQPENNYKTTPPVLDSDGSFFLVSKLTVDKSRWQQGNVFSCSVMHEALHNHYTQKSLSLSP

SEQ ID NO: 32 - protein, 444 aa, Artificial
  An artificially synthesized peptide sequence
QDQLVQSGAEVKKPGASVKVSCKASGFNIKDTYIQWVRQAPGQGLEWMGRIDPLRKQTKYREKFEGRVTITADTSTNTAYMELSSLRSEDTAVYYCVRSGREFDYWGQGTLVTVSSASTKGPSVFPLAPSSKSTSGGTAALGCLVKDYFPEPVTVSWNSGALTSGVHTFPAVLQSSGLYSLSSVVTVPSSSLGTQTYICNVNHKPSNTKVDKKVEPKSCDKTHTCPPCPAPEYQWGPMVFLFPPKPKDTLMISRTPEVTCVVVDVSDEEPEVKFNWYVDGVEVHNAKTKPREEQYNATYRVVSVLTVLHQDWLNGKEYKCKVSNGSGGSPIEKTISKAKGQPREPQVCTLPPSRDELTKNQVSLWCLVKGFYPSDIAVEWESNGQPENNYKTTPPVLDSDGSFFLYSKLTVDKSRWQQGNVFSCSVMHEALHNHYTQKSLSLSP

SEQ ID NO: 33 - protein, 446 aa, Artificial
  An artificially synthesized peptide sequence
QDQLVQSGAEVKKPGASVKVSCKASGFNIKDTYIQWVRQAPGQGLEWMGRIDPLRKQTKYREKFEGRVTITADTSTNTAYMELSSLRSEDTAVYYCVRSGREFDYWGQGTLVTVSSASTKGPSVFPLAPSSKSTSGGTAALGCLVKDYFPEPVTVSWNSGALTSGVHTFPAVLQSSGLYSLSSVVTVPSSSLGTQTYICNVNHKPSNTKVDKKVEPKSCDKTHTCPPCPAPEYQWGPMVFLFPPKPKDTLMISRTPEVTCVVVDVSDEEPEVKFNWYVDGVEVHNAKTKPREEQYNATYRVVSVLTVLHQDWLNGKEYKCKVSNGGSGGGSPIEKTISKAKGQPREPQVCTLPPSRDELTKNQVSLWCLVKGFYPSDIAVEWESNGQPENNYKTTPPVLDSDGSFFLYSKLTVDKSRWQQGNVFSCSVMHEALHNHYTQKSLSLSP

SEQ ID NO: 34 - protein, 450 aa, Artificial
  An artificially synthesized peptide sequence
QDQLVQSGAEVKKPGASVKVSCKASGFNIKDTYIQWVRQAPGQGLEWMGRIDPLRKQTKYREKFEGRVTITADTSTNTAYMELSSLRSEDTAVYYCVRSGREFDYWGQGTLVTVSSASTKGPSVFPLAPSSKSTSGGTAALGCLVKDYFPEPVTVSWNSGALTSGVHTFPAVLQSSGLYSLSSVVTVPSSSLGTQTYICNVNHKPSNTKVDKKVEPKSCDKTHTCPPCPAPEYQWGPMVFLFPPKPKDTLMISRTPEVTCVVVDVSDEEPEVKFNWYVDGVEVHNAKTKPREEQYNATYRVVSVLTVLHQDWLNGKEYKCKVSNGGSGGGSGGGSPIEKTISKAKGQPREPQVCTLPPSRDELTKNQVSLWCLVKGFYPSDIAVEWESNGQPENNYKTTPPVLDSDGSFFLYSKLTVDKSRWQQGNVFSCSVMHEALHNHYTQKSLSLSP

SEQ ID NO: 35 - protein, 447 aa, Artificial
  An artificially synthesized peptide sequence
QDQLVQSGAEVKKPGASVKVSCKASGFNIKDTYIQWVRQAPGQGLEWMGRIDPLRKQTKYREKFEGRVTITADTSTNTAYMELSSLRSEDTAVYYCVRSGREFDYWGQGTLVTVSSASTKGPSVFPLAPSSKSTSGGTAALGCLVKDYFPEPVTVSWNSGALTSGVHTFPAVLQSSGLYSLSSVVTVPSSSLGTQTYICNVNHKPSNTKVDKKVEPKSCDKTHTCPPCPAPEYQWGPMVFLFPPKPKDTLMISRTPEVTCVVVDVSDEGGSEPEVKFNWYVDGVEVHNAKTKPREEQYNATYRVVSVLTVLHQDWLNGKEYKCKVSNKALPAPIEKTISKAKGQPREPQVCTLPPSRDELTKNQVSLWCLVKGFYPSDIAVEWESNGQPENNYKTTPPVLDSDGSFFLYSKLTVDKSRWQQGNVFSCSVMHEALHNHYTQKSLSLSP

SEQ ID NO: 36 - protein, 450 aa, Artificial
  An artificially synthesized peptide sequence
QDQLVQSGAEVKKPGASVKVSCKASGFNIKDTYIQWVRQAPGQGLEWMGRIDPLRKQTKYREKFEGRVTITADTSTNTAYMELSSLRSEDTAVYYCVRSGREFDYWGQGTLVTVSSASTKGPSVFPLAPSSKSTSGGTAALGCLVKDYFPEPVTVSWNSGALTSGVHTFPAVLQSSGLYSLSSVVTVPSSSLGTQTYICNVNHKPSNTKVDKKVEPKSCDKTHTCPPCPAPEYQWGPMVFLFPPKPKDTLMISRTPEVTCVVVDVSDEGGSGGSEPEVKFNWYVDGVEVHNAKTKPREEQYNATYRVVSVLTVLHQDWLNGKEYKCKVSNKALPAPIEKTISKAKGQPREPQVCTLPPSRDELTKNQVSLWCLVKGFYPSDIAVEWESNGQPENNYKTTPPVLDSDGSFFLYSKLTVDKSRWQQGNVFSCSVMHEALHNHYTQKSLSLSP

SEQ ID NO: 37 - protein, 453 aa, Artificial
  An artificially synthesized peptide sequence
QDQLVQSGAEVKKPGASVKVSCKASGFNIKDTYIQWVRQAPGQGLEWMGRIDPLRKQTKYREKFEGRVTITADTSTNTAYMELSSLRSEDTAVYYCVRSGREFDYWGQGTLVTVSSASTKGPSVFPLAPSSKSTSGGTAALGCLVKDYFPEPVTVSWNSGALTSGVHTFPAVLQSSGLYSLSSVVTVPSSSLGTQTYICNVNHKPSNTKVDKKVEPKSCDKTHTCPPCPAPEYQWGPMVFLFPPKPKDTLMISRTPEVTCVVVDVSDEGGSGGSGGSEPEVKFNWYVDGVEVHNAKTKPREEQYNATYRVVSVLTVLHQDWLNGKEYKCKVSNKALPAPIEKTISKAKGQPREPQVCTLPPSRDELTKNQVSLWCLVKGFYPSDIAVEWESNGQPENNYKTTPPVLDSDGSFFLYSKLTVDKSRWQQGNVFSCSVMHEALHNHYTQKSLSLSP

SEQ ID NO: 38 - protein, 447 aa, Artificial
  An artificially synthesized peptide sequence
QDQLVQSGAEVKKPGASVKVSCKASGFNIKDTYIQWVRQAPGQGLEWMGRIDPLRKQTKYREKFEGRVTITADTSTNTAYMELSSLRSEDTAVYYCVRSGREFDYWGQGTLVTVSSASTKGPSVFPLAPSSKSTSGGTAALGCLVKDYFPEPVTVSWNSGALTSGVHTFPAVLQSSGLYSLSSVVTVPSSSLGTQTYICNVNHKPSNTKVDKKVEPKSCDKTHTCPPCPAPEYQWGPMVFLFPPKPKDTLMISRTPEVTCVVVDVSDEEGGSPEVKFNWYVDGVEVHNAKTKPREEQYNATYRVVSVLTVLHQDWLNGKEYKCKVSNKALPAPIEKTISKAKGQPREPQVCTLPPSRDELTKNQVSLWCLVKGFYPSDIAVEWESNGQPENNYKTTPPVLDSDGSFFLYSKLTVDKSRWQQGNVFSCSVMHEALHNHYTQKSLSLSP

SEQ ID NO: 39 - protein, 450 aa, Artificial
  An artificially synthesized peptide sequence
QDQLVQSGAEVKKPGASVKVSCKASGFNIKDTYIQWVRQAPGQGLEWMGRIDPLRKQTKYREKFEGRVTITADTSTNTAYMELSSLRSEDTAVYYCVRSGREFDYWGQGTLVTVSSASTKGPSVFPLAPSSKSTSGGTAALGCLVKDYFPEPVTVSWNSGALTSGVHTFPAVLQSSGLYSLSSVVTVPSSSLGTQTYICNVNHKPSNTKVDKKVEPKSCDKTHTCPPCPAPEYQWGPMVFLFPPKPKDTLMISRTPEVTCVVVDVSDEEGGSGGSPEVKFNWYVDGVEVHNAKTKPREEQYNATYRVVSVLTVLHQDWLNGKEYKCKVSNKALPAPIEKTISKAKGQPREPQVCTLPPSRDELTKNQVSLWCLVKGFYPSDIAVEWESNGQPENNYKTTPPVLDSDGSFFLYSKLTVDKSRWQQGNVFSCSVMHEALHNHYTQKSLSLSP

SEQ ID NO: 40 - protein, 453 aa, Artificial
  An artificially synthesized peptide sequence
QDQLVQSGAEVKKPGASVKVSCKASGFNIKDTYIQWVRQAPGQGLEWMGRIDPLRKQTKYREKFEGRVTITADTSTNTAYMELSSLRSEDTAVYYCVRSGREFDYWGQGTLVTVSSASTKGPSVFPLAPSSKSTSGGTAALGCLVKDYFPEPVTVSWNSGALTSGVHTFPAVLQSSGLYSLSSVVTVPSSSLGTQTYICNVNHKPSNTKVDKKVEPKSCDKTHTCPPCPAPEYQWGPMVFLFPPKPKDTLMISRTPEVTCVVVDVSDEEGGSGGSGGSPEVKFNWYVDGVEVHNAKTKPREEQYNATYRVVSVLTVLHQDWLNGKEYKCKVSNKALPAPIEKTISKAKGQPREPQVCTLPPSRDELTKNQVSLWCLVKGFYPSDIAVEWESNGQPENNYKTTPPVLDSDGSFFLYSKLTVDKSRWQQGNVFSCSVMHEALHNHYTQKSLSLSP

SEQ ID NO: 41 - protein, 447 aa, Artificial
  An artificially synthesized peptide sequence
QDQLVQSGAEVKKPGASVKVSCKASGFNIKDTYIQWVRQAPGQGLEWMGRIDPLRKQTKYREKFEGRVTITADTSTNTAYMELSSLRSEDTAVYYCVRSGREFDYWGQGTLVTVSSASTKGPSVFPLAPSSKSTSGGTAALGCLVKDYFPEPVTVSWNSGALTSGVHTFPAVLQSSGLYSLSSVVTVPSSSLGTQTYICNVNHKPSNTKVDKKVEPKSCDKTHTCPPCPAPEYQWGPMVFLFPPKPKDTLMISRTPEVTCVVVDVSDEEPEVKFNWYVDGVEVHNAKTKPREEQYNATYRVVSVLTVLHQDWLNGKEYKCKVSNKGGSALPAPIEKTISKAKGQPREPQVCTLPPSRDELTKNQVSLWCLVKGFYPSDIAVEWESNGQPENNYKTTPPVLDSDGSFFLYSKLTVDKSRWQQGNVFSCSVMHEALHNHYTQKSLSLSP

SEQ ID NO: 42 - protein, 450 aa, Artificial
  An artificially synthesized peptide sequence
QDQLVQSGAEVKKPGASVKVSCKASGFNIKDTYIQWVRQAPGQGLEWMGRIDPLRKQTKYREKFEGRVTITADTSTNTAYMELSSLRSEDTAVYYCVRSGREFDYWGQGTLVTVSSASTKGPSVFPLAPSSKSTSGGTAALGCLVKDYFPEPVTVSWNSGALTSGVHTFPAVLQSSGLYSLSSVVTVPSSSLGTQTYICNVNHKPSNTKVDKKVEPKSCDKTHTCPPCPAPEYQWGPMVFLFPPKPKDTLMISRTPEVTCVVVDVSDEEPEVKFNWYVDGVEVHNAKTKPREEQYNATYRVVSVLTVLHQDWLNGKEYKCKVSNKGGSGGSALPAPIEKTISKAKGQPREPQVCTLPPSRDELTKNQVSLWCLVKGFYPSDIAVEWESNGQPENNYKTTPPVLDSDGSFFLYSKLTVDKSRWQQGNVFSCSVMHEALHNHYTQKSLSLSP

SEQ ID NO: 43 - protein, 453 aa, Artificial
  An artificially synthesized peptide sequence
QDQLVQSGAEVKKPGASVKVSCKASGFNIKDTYIQWVRQAPGQGLEWMGRIDPLRKQTKYREKFEGRVTITADTSTNTAYMELSSLRSEDTAVYYCVRSGREFDYWGQGTLVTVSSASTKGPSVFPLAPSSKSTSGGTAALGCLVKDYFPEPVTVSWNSGALTSGVHTFPAVLQSSGLYSLSSVVTVPSSSLGTQTYICNVNHKPSNTKVDKKVEPKSCDKTHTCPPCPAPEYQWGPMVFLFPPKPKDTLMISRTPEVTCVVVDVSDEEPEVKFNWYVDGVEVHNAKTKPREEQYNATYRVVSVLTVLHQDWLNGKEYKCKVSNKGGSGGSGGSALPAPIEKTISKAKGQPREPQVCTLPPSRDELTKNQVSLWCLVKGFYPSDIAVEWESNGQPENNYKTTPPVLDSDGSFFLYSKLTVDKSRWQQGNVFSCSVMHEALHNHYTQKSLSLSP

SEQ ID NO: 44 - protein, 444 aa, Homo sapiens
QDQLVQSGAEVKKPGASVKVSCKASGFNIKDTYIQWVRQAPGQGLEWMGRIDPLRKQTKYREKFEGRVTITADTSTNTAYMELSSLRSEDTAVYYCVRSGREFDYWGQGTLVTVSSASTKGPSVFPLAPSSKSTSGGTAALGCLVKDYFPEPVTVSWNSGALTSGVHTFPAVLQSSGLYSLSSVVTVPSSSLGTQTYICNVNHKPSNTKVDKKVEPKSCDKTHTCPPCPAPELLGGPSVFLFPPKPKDTLMISRTPEVTCVVVDVSHEDPEVKFNWYVDGVEVHNAKTKPREEQYNSTYRVVSVLTVLHQDWLNGKEYKCKVSNKALPAPIEKTISKAKGQPREPQVYTLPPSREEMTKNQVSLTCLVKGFYPSDIAVEWESNGQPENNYKTTPPVLDSDGSFFLYSKLTVDKSRWQQGNVFSCSVMHEALHNHYTQKSLSLSP

SEQ ID NO: 45 - protein, 449 aa, Artificial
  An artificially synthesized peptide sequence
QDQLVQSGAEVKKPGASVKVSCKASGFNIKDTYIQWVRQAPGQGLEWMGRIDPLRKQTKYREKFEGRVTITADTSTNTAYMELSSLRSEDTAVYYCVRSGREFDYWGQGTLVTVSSASTKGPSVFPLAPSSKSTSGGTAALGCLVKDYFPEPVTVSWNSGALTSGVHTFPAVLQSSGLYSLSSVVTVPSSSLGTQTYICNVNHKPSNTKVDKKVEPKSCDKTHTCPPCPAPELLGGPSVFLFPPKPKDTLMISRTPEVTCVVVDVSGCRGDCLEPEVKFNWYVDGVEVHNAKTKPREEQYNSTYRVVSVLTVLHQDWLNGKEYKCKVSNDALPMPIEETISKAKGQPREPQVYTLPPSRCELTKNQVSLSCAVKGFYPSDIAVEWESNGQPENNYKTTPPVLDSDGSFFLVSKLTVDKSRWQQGNVFSCSVMHEALHNHYTQKSLSLSP

SEQ ID NO: 46 - protein, 449 aa, Artificial
  An artificially synthesized peptide sequence
QDQLVQSGAEVKKPGASVKVSCKASGFNIKDTYIQWVRQAPGQGLEWMGRIDPLRKQTKYREKFEGRVTITADTSTNTAYMELSSLRSEDTAVYYCVRSGREFDYWGQGTLVTVSSASTKGPSVFPLAPSSKSTSGGTAALGCLVKDYFPEPVTVSWNSGALTSGVHTFPAVLQSSGLYSLSSVVTVPSSSLGTQTYICNVNHKPSNTKVDKKVEPKSCDKTHTCPPCPAPEYQWGPMVFLFPPKPKDTLMISRTPEVTCVVVDVSGCRGDCLEPEVKFNWYVDGVEVHNAKTKPREEQYNATYRVVSVLTVLHQDWLNGKEYKCKVSNKALPAPIEKTISKAKGQPREPQVCTLPPSRDELTKNQVSLWCLVKGFYPSDIAVEWESNGQPENNYKTTPPVLDSDGSFFLYSKLTVDKSRWQQGNVFSCSVMHEALHNHYTQKSLSLSP

SEQ ID NO: 47 - protein, 448 aa, Artificial
  An artificially synthesized peptide sequence
QDQLVQSGAEVKKPGASVKVSCKASGFNIKDTYIQWVRQAPGQGLEWMGRIDPLRKQTKYREKFEGRVTITADTSTNTAYMELSSLRSEDTAVYYCVRSGREFDYWGQGTLVTVSSASTKGPSVFPLAPSSKSTSGGTAALGCLVKDYFPEPVTVSWNSGALTSGVHTFPAVLQSSGLYSLSSVVTVPSSSLGTQTYICNVNHKPSNTKVDKKVEPKSCDKTHTCPPCPAPEYQWGPMVFLFPPKPKDTLMISRTPEVTCVVVDVSDEEPEVKFNWYVDGVEVHNAKTKPREEQYNATYRVVSVLTVLHQDWLNGKEYKCKVSNKALPAPIEKTISKAKGQPREPQVCTLPPSRDELTKNQVSLWCLVKGFYPSDIAVEWESGCRGDCLPENNYKTTPPVLDSDGSFFLYSKLTVDKSRWQQGNVFSCSVMHEALHNHYTQKSLSLSP

SEQ ID NO: 48 - protein, 448 aa, Artificial
  An artificially synthesized peptide sequence
QDQLVQSGAEVKKPGASVKVSCKASGFNIKDTYIQWVRQAPGQGLEWMGRIDPLRKQTKYREKFEGRVTITADTSTNTAYMELSSLRSEDTAVYYCVRSGREFDYWGQGTLVTVSSASTKGPSVFPLAPSSKSTSGGTAALGCLVKDYFPEPVTVSWNSGALTSGVHTFPAVLQSSGLYSLSSVVTVPSSSLGTQTYICNVNHKPSNTKVDKKVEPKSCDKTHTCPPCPAPELLGGPSVFLFPPKPKDTLMISRTPEVTCVVVDVSHEDPEVKFNWYVDGVEVHNAKTKPREEQYNSTYRVVSVLTVLHQDWLNGKEYKCKVSNKALPAPIEKTISKAKGQPREPQVYTLPPSRDELTKNQVSLTCLVKGFYPSDIAVEWESGCRGDCLPENNYKTTPPVLDSDGSFFLYSKLTVDKSRWQQGNVFSCSVMHEALHNHYTQKSLSLSP

SEQ ID NO: 49 - protein, 330 aa, Homo sapiens [sequence omitted]

SEQ ID NO: 50 - protein, 326 aa, Homo sapiens
ASTKGPSVFPLAPCSRSTSESTAALGCLVKDYFPEPVTVSWNSGALTSGVHTFPAVLQSSGLYSLSSVVTVPSSNFGTQTYTCNVDHKPSNTKVDKTVERKCCVECPPCPAPPVAGPSVFLFPPKPKDTLMISRTPEVTCVVVDVSHEDPEVQFNWYVDGVEVHNAKTKPREEQFNSTFRVVSVLTVVHQDWLNGKEYKCKVSNKGLPAPIEKTISKTKGQPREPQVYTLPPSREEMTKNQVSLTCLVKGFYPSDIAVEWESNGQPENNYKTTPPMLDSDGSFFLYSKLTVDKSRWQQGNVFSCSVMHEALHNHYTQKSLSLSPGK

SEQ ID NO: 51 - protein, 377 aa, Homo sapiens
ASTKGPSVFPLAPCSRSTSGGTAALGCLVKDYFPEPVTVSWNSGALTSGVHTFPAVLQSSGLYSLSSVVTVPSSSLGTQTYTCNVNHKPSNTKVDKRVELKTPLGDTTHTCPRCPEPKSCDTPPPCPRCPEPKSCDTPPPCPRCPEPKSCDTPPPCPRCPAPELLGGPSVFLFPPKPKDTLMISRTPEVTCVVVDVSHEDPEVQFKWYVDGVEVHNAKTKPREEQYNSTFRVVSVLTVLHQDWLNGKEYKCKVSNKALPAPIEKTISKTKGQPREPQVYTLPPSREEMTKNQVSLTCLVKGFYPSDIAVEWESSGQPENNYNTTPPMLDSDGSFFLYSKLTVDKSRWQQGNIFSCSVMHEALHNRFTQKSLSLSPGK

SEQ ID NO: 52 - protein, 327 aa, Homo sapiens
ASTKGPSVFPLAPCSRSTSESTAALGCLVKDYFPEPVTVSWNSGALTSGVHTFPAVLQSSGLYSLSSVVTVPSSSLGTKTYTCNVDHKPSNTKVDKRVESKYGPPCPSCPAPEFLGGPSVFLFPPKPKDTLMISRTPEVTCVVVDVSQEDPEVQFNWYVDGVEVHNAKTKPREEQFNSTYRVVSVLTVLHQDWLNGKEYKCKVSNKGLPSSIEKTISKAKGQPREPQVYTLPPSQEEMTKNQVSLTCLVKGFYPSDIAVEWESNGQPENNYKTTPPVLDSDGSFFLYSRLTVDKSRWQEGNVFSCSVMHEALHNHYTQKSLSLSLGK

SEQ ID NO: 53 - protein, 230 aa, Artificial
  An artificially synthesized peptide sequence
EPKSSDKTHTCPPCPAPELLGGPDVFLFPPKPKDTLMISRTPEVTCVVVDVSHEDPEVKFNWYVDGVEVHNAKTKPREEQYNSTYRVVSVLTVLHQDWLNGKEYKCKVSNKALPLPEEKTISKAKGQPREPQVCTLPPSRDELTKNQVSLWCLVKGFYPSDIAVEWESNGQPENNYKTTPPVLDSDGSFFLYSKLTVDKSRWQQGNVFSCSVMHEALHNHYTQKSLSLSP

SEQ ID NO: 54 - protein, 230 aa, Artificial
  An artificially synthesized peptide sequence
EPKSSDKTHTCPPCPAPEYLWGPSVFLFPPKPKDTLMISRTPEVTCVVVDVSHEDPEVKFNWYVDGVEVHNAKTKPREEQYNATYRVVSVLTVLHQDWLNGKEYKCKVSNKALPAPIEKTISKAKGQPREPQVYTLPPSRCELTKNQVSLSCAVKGFYPSDIAVEWESNGQPENNYKTTPPVLDSDGSFFLVSKLTVDKSRWQQGNVFSCSVMHEALHNHYTQKSLSLSP